European Patent Specification EP 4 217 398 B1, published September 24, 2025. Title: ANTI-C-MET ANTIBODY DRUG CONJUGATES. Applicant: AbbVie Inc. The sequence listing filed with the application follows.

SEQUENCE LISTING (28 sequences)

SEQ ID NO: 1 - protein, 8 aa, Artificial Sequence
  Synthetic polypeptide
GYIFTAYT

SEQ ID NO: 2 - protein, 8 aa, Artificial Sequence
  Synthetic polypeptide
IKPNNGLA

SEQ ID NO: 3 - protein, 11 aa, Artificial Sequence
  Synthetic polypeptide
ARSEITTEFDY

SEQ ID NO: 4 - protein, 10 aa, Artificial Sequence
  Synthetic polypeptide
ESVDSYANSF

SEQ ID NO: 5 - protein, 3 aa, Artificial Sequence
  Synthetic polypeptide
RAS

SEQ ID NO: 6 - protein, 9 aa, Artificial Sequence
  Synthetic polypeptide
QQSKEDPLT

SEQ ID NO: 7 - protein, 118 aa, Artificial Sequence
  Synthetic polypeptide
QVQLVQSGAEVKKPGASVKVSCKASGYIFTAYTMHWVRQAPGQGLEWMGWIKPNNGLANYAQKFQGRVTMTRDTSISTAYMELSRLRSDDTAVYYCARSEITTEFDYWGQGTLVTVSS

SEQ ID NO: 8 - protein, 111 aa, Artificial Sequence
  Synthetic polypeptide
DIVMTQSPDSLAVSLGERATINCKSSESVDSYANSFLHWYQQKPGQPPKLLIYRASTRESGVPDRFSGSGSGTDFTLTISSLQAEDVAVYYCQQSKEDPLTFGGGTKVEIK

SEQ ID NO: 9 - protein, 445 aa, Artificial Sequence
  Synthetic polypeptide
QVQLVQSGAEVKKPGASVKVSCKASGYIFTAYTMHWVRQAPGQGLEWMGWIKPNNGLANYAQKFQGRVTMTRDTSISTAYMELSRLRSDDTAVYYCARSEITTEFDYWGQGTLVTVSSASTKGPSVFPLAPSSKSTSGGTAALGCLVKDYFPEPVTVSWNSGALTSGVHTFPAVLQSSGLYSLSSVVTVPSSSLGTQTYICNVNHKPSNTKVDKRVEPKSCDCHCPPCPAPELLGGPSVFLFPPKPKDTLMISRTPEVTCVVVDVSHEDPEVKFNWYVDGVEVHNAKTKPREEQYNSTYRVVSVLTVLHQDWLNGKEYKCKVSNKALPAPIEKTISKAKGQPREPQVYTLPPSREEMTKNQVSLTCLVKGFYPSDIAVEWESNGQPENNYKTTPPVLDSDGSFFLYSKLTVDKSRWQQGNVFSCSVMHEALHNHYTQKSLSLSPG

SEQ ID NO: 10 - protein, 218 aa, Artificial Sequence
  Synthetic polypeptide
DIVMTQSPDSLAVSLGERATINCKSSESVDSYANSFLHWYQQKPGQPPKLLIYRASTRESGVPDRFSGSGSGTDFTLTISSLQAEDVAVYYCQQSKEDPLTFGGGTKVEIKRTVAAPSVFIFPPSDEQLKSGTASVVCLLNNFYPREAKVQWKVDNALQSGNSQESVTEQDSKDSTYSLSSTLTLSKADYEKHKVYACEVTHQGLSSPVTKSFNRGEC

SEQ ID NO: 11 - protein, 460 aa, Artificial Sequence
  Synthetic polypeptide
EEQVLESGGGLVKPGGSLRLSCAASGFTFSPYSVFWVRQAPGKGLEWVSSINSDSTYKYYADSVKGRFTISRDNAENSIFLQMNSLRAEDTAVYYCARDRSYYAFSSGSLSDYYYGLDVWGQGTTVIVSSASTKGPSVFPLAPSSKSTSGGTAALGCLVKDYFPEPVTVSWNSGALTSGVHTFPAVLQSSGLYSLSSVVTVPSSSLGTQTYICNVNHKPSNTKVDKKVEPKSCDKTHTCPPCPAPEAAGGPSVFLFPPKPKDTLMISRTPEVTCVVVDVSHEDPEVKFNWYVDGVEVHNAKTKPREEQYNSTYRVVSVLTVLHQDWLNGKEYKCKVSNKALPAPIEKTISKAKGQPREPQVYTLPPSRDELTKNQVSLTCLVKGFYPSDIAVEWESNGQPENNYKTTPPVLDSDGSFFLYSKLTVDKSRWQQGNVFSCSVMHEALHNHYTQKSLSLSPGK

SEQ ID NO: 12 - protein, 219 aa, Artificial Sequence
  Synthetic polypeptide
DIVMTQSPLSLSVTPGEPASISCRSSQSLLHTNGYNYLDWYVQKPGQSPQLLIYLASNRASGVPDRFSGSGSGTDFTLKISRVETEDVGVYYCMQALQIPRTFGQGTKVEIKRTVAAPSVFIFPPSDEQLKSGTASVVCLLNNFYPREAKVQWKVDNALQSGNSQESVTEQDSKDSTYSLSSTLTLSKADYEKHKVYACEVTHQGLSSPVTKSFNRGEA

SEQ ID NO: 13 - protein, 118 aa, Artificial Sequence
  Synthetic polypeptide
EVQLQQSGPELVKPGASVKISCKTSGYIFTAYTMHWVRQSLGESLDWIGGIKPNNGLANYNQKFKGKATLTVDKSSSTAYMDLRSLTSEDSAVYYCARSEITTEFDYWGQGTALTVSS

SEQ ID NO: 14 - protein, 111 aa, Artificial Sequence
  Synthetic polypeptide
DIVLTQSPASLAVSLGQRATISCRASESVDSYANSFMHWYQQKPGQPPKLLIYRASNLESGIPARFSGSGSRTDFTLTINPVEADDVATYYCQQSKEDPLTFGSGTKLEMK

SEQ ID NO: 15 - protein, 8 aa, Artificial Sequence
  Synthetic polypeptide
GYIFTAYT

SEQ ID NO: 16 - protein, 8 aa, Artificial Sequence
  Synthetic polypeptide
IKPNNGLA

SEQ ID NO: 17 - protein, 11 aa, Artificial Sequence
  Synthetic polypeptide
ARSEITTEFDY

SEQ ID NO: 18 - protein, 10 aa, Artificial Sequence
  Synthetic polypeptide
ESVDSYANSF

SEQ ID NO: 19 - protein, 3 aa, Artificial Sequence
  Synthetic polypeptide
RAS

SEQ ID NO: 20 - protein, 9 aa, Artificial Sequence
  Synthetic polypeptide
QQSKEDPLT

SEQ ID NO: 21 - DNA, 1395 bp, Artificial Sequence
  Synthetic polynucleotide
atgggatggtcttggatctttctgctgtttctgtctggtactgctggtgtgctgagccaggtccagctggtgcaatccggcgcagaggtgaagaagccaggcgcttccgtgaaggtgagctgtaaggcctctggctacatcttcacagcatacaccatgcactgggtgaggcaagctcctgggcagggactggagtggatgggatggattaaacccaacaatgggctggccaactacgcccagaaattccagggtagggtcactatgacaagggataccagcatcagcaccgcatatatggagctgagcaggctgaggtctgacgacactgctgtctattattgcgccaggagcgaaattacaacagaattcgattactgggggcagggcaccctggtgaccgtgtcctctgccagcaccaagggcccaagcgtgttccccctggcccccagcagcaagagcaccagcggcggcacagccgccctgggctgcctggtgaaggactacttccccgagcccgtgaccgtgtcctggaacagcggagccctcacttctggagttcataccttcccagcagtattgcagagcagtggcctgtattcactgtcttccgtcgtaacagttccatcctccagcctcgggacacagacttacatttgtaacgtgaatcacaagcctagcaacaccaaggtcgacaagagagttgaaccaaagagttgtgattgccactgtcctccctgcccagctcctgagctgcttggcggtcccagtgtcttcttgtttccccctaaacccaaagacaccctgatgatctcaaggactcccgaggtgacatgcgtggtggtggatgtgtctcatgaggacccagaggtgaagttcaactggtacgtggacggcgtggaggtgcacaacgccaagaccaagcccagagaggagcagtacaacagcacctacagggtggtgtccgtgctgaccgtgctgcaccaggactggctgaacggcaaggagtacaagtgtaaggtgtccaacaaggccctgccagccccaatcgaaaagaccatcagcaaggccaagggccagccaagagagccccaggtgtacaccctgccacccagcagggaggagatgaccaagaaccaggtgtccctgacctgtctggtgaagggcttctacccaagcgacatcgccgtggagtgggagagcaacggccagcccgagaacaactacaagaccacccccccagtgctggacagcgacggcagcttcttcctgtacagcaagctgaccgtggacaagagcagatggcagcagggcaacgtgttcagctgctccgtgatgcacgaggccctgcacaaccactacacccagaagagcctgagcctgtccccaggctga

SEQ ID NO: 22 - DNA, 24 bp, Artificial Sequence
  Synthetic polynucleotide
ggctacatcttcacagcatacacc

SEQ ID NO: 23 - DNA, 24 bp, Artificial Sequence
  Synthetic polynucleotide
attaaacccaacaatgggctggcc

SEQ ID NO: 24 - DNA, 33 bp, Artificial Sequence
  Synthetic polynucleotide
gccaggagcgaaattacaacagaattcgattac

SEQ ID NO: 25 - DNA, 717 bp, Artificial Sequence
  Synthetic polynucleotide
atggaaactgatacactgctgctgtgggtcctgctgctgtgggtccctggaagcacaggggacattgtgatgacccagtctcccgatagcctggccgtgtccctgggcgagagggctaccatcaactgtaaaagctccgaatctgtggactcttacgcaaacagctttctgcactggtatcagcaaaagccaggccaacctccaaagctgctgatttacagggcttctaccagggagagcggcgtgcccgataggttcagcggatctggcagcggcaccgactttacactgaccatctccagcctgcaggccgaagatgtggcagtctattactgccagcagtccaaggaggaccccctgactttcgggggtggtactaaagtggagatcaagcgtacggtggccgctcccagcgtgttcatcttccccccaagcgacgagcagctgaagagcggcaccgccagcgtggtgtgtctgctgaacaacttctaccccagggaggccaaggtgcagtggaaggtggacaacgccctgcagagcggcaacagccaggagagcgtcaccgagcaggacagcaaggactccacctacagcctgagcagcaccctgaccctgagcaaggccgactacgagaagcacaaggtgtacgcctgtgaggtgacccaccagggcctgtccagccccgtgaccaagagcttcaacaggggcgagtgctga

SEQ ID NO: 26 - DNA, 30 bp, Artificial Sequence
  Synthetic polynucleotide
gaatctgtggactcttacgcaaacagcttt

SEQ ID NO: 27 - DNA, 9 bp, Artificial Sequence
  Synthetic polynucleotide
agggcttct

SEQ ID NO: 28 - DNA, 27 bp, Artificial Sequence
  Synthetic polynucleotide
cagcagtccaaggaggaccccctgact